European Patent Specification EP 3 645 559 B1, published December 4, 2024. Title: Pharmaceuticals and devices for the immobilization of IGF-1's D domain and derivatives thereof to extracellular matrices by human transglutaminase. Applicant: Julius-Maximilians-Universität Würzburg. The sequence listing filed with the application follows.

SEQUENCE LISTING (12 sequences)

SEQ ID NO: 1 - protein, 8 aa, Homo sapiens
PLKPAKSA

SEQ ID NO: 2 - protein, 7 aa, Homo sapiens
LKPAKSA

SEQ ID NO: 3 - protein, 6 aa, Homo sapiens
KPAKSA

SEQ ID NO: 4 - protein, 5 aa, Homo sapiens
PAKSA

SEQ ID NO: 5 - protein, 4 aa, Homo sapiens
AKSA

SEQ ID NO: 6 - protein, 8 aa, Mus musculus
PLKPTKAA

SEQ ID NO: 7 - protein, 7 aa, Mus musculus
LKPTKAA

SEQ ID NO: 8 - protein, 6 aa, Mus musculus
KPTKAA

SEQ ID NO: 9 - protein, 5 aa, Mus musculus
PTKAA

SEQ ID NO: 10 - protein, 4 aa, Mus musculus
TKAA

SEQ ID NO: 11 - protein, 8 aa, Homo sapiens
NQEQVSPL

SEQ ID NO: 12 - protein, 8 aa, Synthetic sequence (mutant IGF-I D-Domain)
PLKPARSA